European Patent Application EP 4 714 963 A1, published March 25, 2026. Title: peptide fragment and use thereof. Applicant: TOAGOSEI CO., LTD. The sequence listing filed with the application follows.

SEQUENCE LISTING (8 sequences)

SEQ ID NO: 1 - protein, 9 aa, synthetic construct
RRRRSNRRG

SEQ ID NO: 2 - protein, 7 aa, synthetic construct
RRRRRRG

SEQ ID NO: 3 - protein, 9 aa, synthetic construct
SNRRRRRRG

SEQ ID NO: 4 - protein, 9 aa, synthetic construct
RSNRRRRRG

SEQ ID NO: 5 - protein, 9 aa, synthetic construct
RRSNRRRRG

SEQ ID NO: 6 - protein, 9 aa, synthetic construct
RRRSNRRRG

SEQ ID NO: 7 - protein, 9 aa, synthetic construct
RRRRRSNRG

SEQ ID NO: 8 - protein, 9 aa, synthetic construct
RRRRRRSNG